European Patent Application EP 4 691 490 A1, published February 11, 2026. Title: PHARMACEUTICAL COMPOSITION FOR TREATMENT AND/OR PREVENTION OF CANCER. Applicant: TORAY Industries, Inc. The sequence listing filed with the application follows.

SEQUENCE LISTING (4 sequences)

SEQ ID NO: 1 - DNA, 18 bp, synthetic construct
  source 1..18: mol_type = other DNA
aaggtttgaatggagtgc

SEQ ID NO: 2 - DNA, 18 bp, synthetic construct
  source 1..18: mol_type = other DNA
tgctccttttcaccactg

SEQ ID NO: 3 - DNA, 18 bp, synthetic construct
  source 1..18: mol_type = other DNA
gggctgcttttaactctg

SEQ ID NO: 4 - DNA, 18 bp, synthetic construct
  source 1..18: mol_type = other DNA
tgctccttttcaccactg